European Patent Application EP 4 631 961 A1, published October 15, 2025. Title: Peptide for cartilage regeneration and uses thereof. Applicant: CAREGEN CO., LTD. The sequence listing filed with the application follows.

SEQUENCE LISTING (15 sequences)

SEQ ID NO: 1 - protein, 9 aa, synthetic construct
LYRYEEHHE

SEQ ID NO: 2 - DNA, 23 bp, synthetic construct
  source 1..23: mol_type = other DNA
ctatctggacgaagcagctggca

SEQ ID NO: 3 - DNA, 22 bp, synthetic construct
  source 1..22: mol_type = other DNA
atgggtgcaatgtcaatgatgg

SEQ ID NO: 4 - DNA, 20 bp, synthetic construct
  source 1..20: mol_type = other DNA
aactcagggcaggaggatgt

SEQ ID NO: 5 - DNA, 20 bp, synthetic construct
  source 1..20: mol_type = other DNA
tgtccttttggtcgtcgttc

SEQ ID NO: 6 - DNA, 20 bp, synthetic construct
  source 1..20: mol_type = other DNA
ccagcccgaacttgtaaaga

SEQ ID NO: 7 - DNA, 20 bp, synthetic construct
  source 1..20: mol_type = other DNA
tggacgcacaaccatcatac

SEQ ID NO: 8 - DNA, 20 bp, synthetic construct
  source 1..20: mol_type = other DNA
tgagtcctcaagcctcctgt

SEQ ID NO: 9 - DNA, 20 bp, synthetic construct
  source 1..20: mol_type = other DNA
gtgccagatcatcaccacac

SEQ ID NO: 10 - DNA, 20 bp, synthetic construct
  source 1..20: mol_type = other DNA
gcaggctatgagcagtgtga

SEQ ID NO: 11 - DNA, 20 bp, synthetic construct
  source 1..20: mol_type = other DNA
gcatacctcggaagcagaag

SEQ ID NO: 12 - DNA, 20 bp, synthetic construct
  source 1..20: mol_type = other DNA
accacagtccatgccatcac

SEQ ID NO: 13 - DNA, 20 bp, synthetic construct
  source 1..20: mol_type = other DNA
tccaccaccctgttgctgta

SEQ ID NO: 14 - DNA, 20 bp, synthetic construct
  source 1..20: mol_type = other DNA
gcggaggaagtcggtgaaga

SEQ ID NO: 15 - DNA, 20 bp, synthetic construct
  source 1..20: mol_type = other DNA
ccctctcgcttcaggtcagc